European Patent Application EP 4 485 463 A1, published January 1, 2025. Title: Modeling enhancers using machine-learning. Applicant: Shape Therapeutics Inc. Application EP. The sequence listing filed with the application follows.

SEQUENCE LISTING (10 sequences)

SEQ ID NO: 1 - DNA, 10 bp, synthetic construct
  source 1..10: mol_type = other DNA
atgccaggaa

SEQ ID NO: 2 - DNA, 10 bp, synthetic construct
  source 1..10: mol_type = other DNA
ttcctggcat

SEQ ID NO: 3 - DNA, 10 bp, synthetic construct
  source 1..10: mol_type = other DNA
agtatggccg

SEQ ID NO: 4 - DNA, 10 bp, synthetic construct
  source 1..10: mol_type = other DNA
atatcggccg

SEQ ID NO: 5 - DNA, 10 bp, synthetic construct
  source 1..10: mol_type = other DNA
agagtacccg

SEQ ID NO: 6 - DNA, 10 bp, synthetic construct
  source 1..10: mol_type = other DNA
atgccaggaa

SEQ ID NO: 7 - DNA, 11 bp, synthetic construct
  source 1..11: mol_type = other DNA
caaagttgagc

SEQ ID NO: 8 - DNA, 11 bp, synthetic construct
  source 1..11: mol_type = other DNA
caaaggtggcc

SEQ ID NO: 9 - DNA, 11 bp, synthetic construct
  source 1..11: mol_type = other DNA
gatctacactg

SEQ ID NO: 10 - DNA, 11 bp, synthetic construct
  source 1..11: mol_type = other DNA
tggccatatct